European Patent Specification EP 4 062 929 B1, published July 9, 2025. Title: Cross-linked Abeta which can be an ASPD substitute, and analysis of ASPD. Applicant: TAO HEALTH LIFE PHARMA CO., LTD. The sequence listing filed with the application follows.

SEQUENCE LISTING (4 sequences)

SEQ ID NO: 1 - protein, 120 aa, Artificial Sequence
  humanized antibody
EVQLVESGGGLVKPGGSLRLSCAASGFTFSDYFMSWVRQAPGKGLEWVGGIEIKSYFYATYYFGSVKGRFTISRDDSKNTLYLQMNSLKTEDTAVYYCTTNREVGGLDNWGQGTLVTVSS

SEQ ID NO: 2 - protein, 117 aa, Artificial Sequence
  humanized antibody
QSVLTQPSSLSASPGASASLTCTLRSGISVGGKNIYWYQQKPGSPPQYLLKYSSYSNKQLGPGVPSRFSGSKDASANAGILLISGLQSEDEADYYCSIHESNAYVFGGGTKLTVLGR

SEQ ID NO: 3 - protein, 120 aa, Artificial Sequence
  recombinant antibody
  Xaa (49)..(49): Gly or Ala
  Xaa (81)..(81): Leu or Val
  Xaa (100)..(100): Thr or Arg
EVQLVESGGGLVKPGGSLRLSCAASGFTFSDYFMSWVRQAPGKGLEWVXGIEIKSYFYATYYFGSVKGRFTISRDDSKNTXYLQMNSLKTEDTAVYYCTXNREVGGLDNWGQGTLVTVSS

SEQ ID NO: 4 - protein, 116 aa, Artificial Sequence
  recombinant antibody
  Xaa (2)..(2): Ser or Ala
  Xaa (8)..(8): Ser or Ala
  Xaa (48)..(48): Tyr or Phe
  Xaa (49)..(49): Leu or Phe
  Xaa (51)..(51): Lys, Phe or Arg
  Xaa (74)..(74): Ala or Thr
  Xaa (79)..(79): Gly or Ala
QXVLTQPXSLSASPGASASLTCTLRSGISVGGKNIYWYQQKPGSPPQXXLXYSSYSNKQLGPGVPSRFSGSKDXSANAXILLISGLQSEDEADYYCSIHESNAYVFGGGTKLTVLG